European Patent Application EP 4 789 534 A1, published August 12, 2026. Title: Method of producing plants with controlled stomatal density and use thereof. Applicant: KYUSHU UNIVERSITY, NATIONAL UNIVERSITY CORPORATION. Application JP. The sequence listing filed with the application follows.

SEQUENCE LISTING (7 sequences)

SEQ ID NO: 1 - protein, 894 aa, Oryza sativa
MPPWWGKSFSKDAKKTTKENLIDTFHRLISPNDQKGSTKSKRSCRRGNDSSVEKSCRSTTVSRPTSPSKEVSRCQSFSADRPHAHPLPIPGVRPPVTRTVSDITESKPILEKRGKPPLLLPLPKPNRPPRRHGNSEVVSEIVVASPSSNCSDSDDHGDSQLQSPVGNDAENATLVTLKNKSSNARKECPGPITAKNMKEIHRPANQVHGSHILSTSPRGVAADSYQSNLQNPRPLVLDSAPNSLMSSPSRSPRRICPDHIPTSAFWAVKPHTDVTFVGSGQCSSPGSGQTSGHNSVGGDMLAQLFWQPSRSSPECSPIPSPRMTSPGPSSRVHSGSVSPLHPRSGGMAPESPTNRHDDGKKKQTHKLPLPPLSISHSSFHPNNSTPTSPISVPRSPGRTENPPSPGSRWKKGKLIGRGTFGHVYVGFNSDSGEMCAMKEVTLFLDDPKSKESAKQLGQEISLLSRLQHPNIVQYYGSETVDDKLYIYLEYVSGGSIHKLLQEYGQLGEQAIRSYTQQILSGLAYLHAKNTVHRDIKGANILVDPSGRVKLADFGMAKHINGQQCPFSFKGSPYWMAPEVIKNSNGCNLAVDIWSLGCTVLEMATSKPPWSQYEGIAAMFKIGNSKELPPIPDHLSEPGKDFIRKCLQRDPSQRPTAMELLQHPFVQKAVSLEKSVLSEPLEHLAVISCRSSAKMAAHTRNISSLGLEGQTIYQRRGAKFSSKHSDIRIRSNISCPVSPCGSPLLKSRSPQHSNGRMSPSPISSPRTTSGTSTPLSGGNGAIPFNHLKQSTYSNEGFAIPSRSPDDLFASRPTDPDLGQFIRVHQVSQGLQERVVSEADILSPQFGKRLGNVFDLRDKLSPSERFTHHAFVDHVKLNPSLDLTSGSPHLGLKHGN

SEQ ID NO: 2 - DNA, 154 bp, Oryza sativa
  source 1..154: mol_type = genomic DNA
caaaagatggtggctagatgatctgggttaaaaacctcatcccttctaattatttgatattatatcattctctaatattcgcgtcttttttaaatcgatgaatgatgaaatgacatcccttttcttttgtgtagcgagtgaaagtgtagtactt

SEQ ID NO: 3 - DNA, 254 bp, Oryza sativa
  source 1..254: mol_type = genomic DNA
tcggtttaattgtacaccgaatcaccaattaaattcaactctttttattttttttagattttatagatccaacaaaaaaatttatagaggagttcatcataattgctctttgacattttgttaaaaagttaatctaaaatgtttgccgtcgtacaattgtgaaaggtctatttagaacaaaggtattaaaacacaaaaatattagaaacatttctcatacacaaataatagtaacgataggcatgctgatggca

SEQ ID NO: 4 - DNA, 157 bp, Oryza sativa
  source 1..157: mol_type = genomic DNA
aacggaccgtctcgatgaagctaccgtagtccgtagcaacggcgccttatatacatcccctccatatcgaggctcgaagcgtactcggtactgcggtagcacgcctgggaacacagaacacagggggaaaaaaagaaccgttgctaccccgatgcgc

SEQ ID NO: 5 - DNA, 180 bp, Lactuca sativa
  source 1..180: mol_type = genomic DNA
taacgacttaccccactagtacaagtccactctcttctcctccattaaacaaatctaaagtgaaagcaaaaaagagaacccaacccctcctcctcctctctctatactttctccgatctctctctcttgctctccttttcccagtttattctcacagaacatcacttggaaacctcacaa

SEQ ID NO: 6 - DNA, 194 bp, Arabidopsis thaliana
  source 1..194: mol_type = genomic DNA
gtggtcaaaacaccaatgggataataataaaatggtgtttatattgggacttttcttcgtttgttgacctatgttgggtcaaccaagtatgatctctgaagtggtcaaaaggagagttactttgtaatgttgaacaagagcttttaaaagagtgatagtgtgagtgagtgtgcctcttggtttgtgggaagaag

SEQ ID NO: 7 - DNA, 173 bp, Hordeum vulgare
  source 1..173: mol_type = genomic DNA
aatcccaaagccacgggtcaaccagaccccaacccggtccagcaccgagttccctcgagccttgcagtttgcggttggaaggcagaggggatcgatcccggcaggcgagccgcggcgatcgtgtggcggttgccgctttgcctcagtttccactgctgtgtctgtgtgtgtgg